European Patent Application EP 4 732 827 A1, published April 29, 2026. Title: MULTIPLE CERAMIDES COMPOSITION AND USE THEREOF. Applicant: LCS Biotech Co., Ltd. Application EP. The sequence listing filed with the application follows.

SEQUENCE LISTING (12 sequences)

SEQ ID NO: 1 - DNA, 22 bp, Artificial Sequence
  source 1..22: mol_type = other DNA
acattccacaaggcaaccattg

SEQ ID NO: 2 - DNA, 20 bp, Artificial Sequence
  source 1..20: mol_type = other DNA
ctcttgattccgccgactcc

SEQ ID NO: 3 - DNA, 20 bp, Artificial Sequence
  source 1..20: mol_type = other DNA
gcgcgctacttggagaaaga

SEQ ID NO: 4 - DNA, 20 bp, Artificial Sequence
  source 1..20: mol_type = other DNA
tgttccaccgtgaccacaac

SEQ ID NO: 5 - DNA, 20 bp, Artificial Sequence
  source 1..20: mol_type = other DNA
tagtgtccacggcactcaac

SEQ ID NO: 6 - DNA, 20 bp, Artificial Sequence
  source 1..20: mol_type = other DNA
aagtaccaccacagagcagc

SEQ ID NO: 7 - DNA, 20 bp, Artificial Sequence
  source 1..20: mol_type = other DNA
ggcactgaaaggcaaaaagg

SEQ ID NO: 8 - DNA, 22 bp, Artificial Sequence
  source 1..22: mol_type = other DNA
aaacccggattcaccataatca

SEQ ID NO: 9 - DNA, 22 bp, Artificial Sequence
  source 1..22: mol_type = other DNA
ccatcaggagcaaatgaaacag

SEQ ID NO: 10 - DNA, 19 bp, Artificial Sequence
  source 1..19: mol_type = other DNA
gctcgacaggcaccttctg

SEQ ID NO: 11 - DNA, 22 bp, Artificial Sequence
  source 1..22: mol_type = other DNA
gacctggatgctctggaacaca

SEQ ID NO: 12 - DNA, 19 bp, Artificial Sequence
  source 1..19: mol_type = other DNA
gaatcgatggcctgctgga